European Patent Application EP 4 389 865 A1, published June 26, 2024. Title: RECOMBINANT PROTEASE FOR CELL DETACHMENT. Applicant: Novozymes A/S. Application EP. The sequence listing filed with the application follows.

SEQUENCE LISTING (3 sequences)

SEQ ID NO: 1 - protein, 223 aa, Paralithodes camtschaticus
QLSFQDTSFGGEFHFCGASIYKDTWAICAGHCVQGEDMNNPDYLQVVAGEFDLDTEESTEQTVILSKIIQHEDYNGFTISNDISLLQFSEPLAFNEFVAAIDLPAQGHAASGDCICSGWGALTEGGSSPSTLYKVTVPIVSDADCRVSYGESEIDDSMICAGVPEGGKDACQGDSGGPLACSDTGSPYLAGIVSWGYGCARPDYPGVYAEVAYFVDWVLANSS

SEQ ID NO: 2 - DNA, 810 bp, synthetic construct
  source 1..810: mol_type = other DNA
  sig_peptide 1..57
  propeptide 58..99
  mat_peptide 142..810
atgaagctctcctggttggtcgcagcagccttgacagccgcatccgtggtctccgcagctccgtcccgcaagcccacctttcgccgaggccttaacaagatcgtcggaggcaccgaggttacccctggggagatcccctaccagttgtcattccaagacacctcctttggtggcgagttccacttctgtggtgcctcgatctacaaagatacttgggccatttgtgctggccactgcgtgcagggcgaagatatgaacaatcccgactacctccaagtggtcgcaggcgagttcgatctggatactgaagaatccaccgaacagaccgtcatcctcagtaagatcatccaacacgaggattacaacggctttaccatctccaacgacatcagccttcttcagtttagcgagcctctcgcctttaacgagtttgttgctgccattgatctgcctgcgcagggccatgctgcgtctggcgattgcatctgctccggctggggtgcgcttaccgaaggtgggagctcccctagcactctgtacaaggtgaccgttcccatcgtgagcgacgccgactgtcgtgtctcgtatggggaatcggagattgatgactcgatgatttgtgccggagtccctgagggtgggaaggacgcctgccagggcgattcaggaggtcccctcgcctgctccgacacaggcagcccttacctcgctggcattgtctcatgggggtacggttgtgctcgtcccgactatcccggtgtatacgccgaggtcgcttacttcgtggactgggtcctggcaaactcgtcc

SEQ ID NO: 3 - protein, 19 aa, Aspergillus aculeatus
MKLSWLVAAALTAASVVSA